European Patent Application EP 4 257 606 A1, published October 11, 2023. Title: PREPARATION AND USE OF ANTI-FSHR ANTIBODY AND ANTIBODY-DRUG CONJUGATE THEREOF. Applicant: CANWELL BIOTECH LIMITED. The sequence listing filed with the application follows.

SEQUENCE LISTING (14 sequences)

SEQ ID NO: 1 - DNA, 714 bp, Artificial Sequence
  Light chain DNA sequence
atggccctccctgtcaccgccctgctgcttccgctggctcttctgctccacgccgctcggccccagatagtacttacgcaatcacccgtcataatgagcgcatcccctggtgaaaaggttactctgacatgctctgcgtcttccagcgtgagtagttcttatctctattggtatcagcaaaaacccggatcttctagtaaattgtggatatattctacgtctaatcttgcgtcaggagtgcctgctcggttttctgggtccgggtccgggaccagctatagtttgactataagtagtatggaggcggaggacgcagctagctacttttgccatcaatggagctcctatcctcctacctttgggggcggaaccaaattggaaatcaaaagagccgacgcggcacccactgtatctatcttcccaccctcatcagaacagctcacttcaggcggcgccagtgtggtgtgtttcctcaacaacttctatcctaaagacataaatgtaaaatggaaaatagacggtagcgagcggcaaaacggggtgctgaactcatggacggaccaagattccaaggattctacctattcaatgagttctacattgacacttacgaaagacgaatacgagcgccacaattcctatacgtgcgaagcaacgcacaaaacctccacttccccgattgtgaagtccttcaataggaatgaatgttgataa

SEQ ID NO: 2 - DNA, 1404 bp, Artificial Sequence
  Heavy chain DNA sequence
atggagtttgggctcagttgggtctttctcgtggcactgtttcgcggggtacagtgcgctagccaagtacaactgcaacaaccaggcgcggagctcgttaaaccgggggcgagcgtcaaccttagctgcaaagcctccggttatacctttacaagttactggatgcactgggtgaagcagcgaccagggcaaggacgcgaatggatcggggaaataaatccaaggaacggcagaacgaattacaacgagaagttcaaatccaaggcgacgttgacggtggacaaatcctcttcaactgcttatatgcagctcagttctctgacaagcgaggatagtgccgtgtactgttgcgccaggttgtctgtggggttcgcctactgggggcagggcacgctcgttacagtctctgcggccaagacgactgcgccttcagtatatccactggctccggtgtgcggagatacgacaggtagttctgtaactttgggatgcctcgttaagggttatttcccggagccggtcaccttgacgtggaactccggatcactctcctcaggggtacatacatttccagcggttttgcagagcgacctctacacactcagtagcagtgtaaccgttacctcatccacatggcctagccagagtatcacgtgcaatgttgcacacccggcaagttctaccaaggtggacaaaaaactcgagcctagaggaccgacgataaagccctgtccgccttgcaaatgtccggcacctaacgctgctggtggcccctctgtttttatatttccgccaaaaattaaggacgtcctcatgatcagtctgagccctatagtcacgtgtgtggtggtagatgtctctgaagacgatcccgacgtacagatttcatggttcgtgaacaatgtggaggttcacacagcccaaacacagacacaccgcgaagattacaatagtacactgcgggtagtctctgccctcccaatacaacaccaggactggatgagcgggaaagagttcaagtgcaaagtcaataacaaagacctgggagcgccgatagaaagaactataagtaaaccaaaggggagcgtaagagcgccccaagtgtatgtcctccctcctcccgaagaggaaatgaccaagaaacaagttactctcacatgcatggtaaccgatttcatgcctgaagacatatacgtagagtggaccaacaacgggaagacagaattgaactacaagaatacagagcccgttctcgattctgatggctcctactttatgtatagcaaactccgggtggaaaaaaagaattgggtcgaaagaaacagttattcatgttctgttgttcacgagggtttgcataaccatcatacgacgaaatctttttccagaaccccaggaaaatga

SEQ ID NO: 3 - protein, 236 aa, Artificial Sequence
  Light chain amino acid sequence
MALPVTALLLPLALLLHAARPQIVLTQSPVIMSASPGEKVTLTCSASSSVSSSYLYWYQQKPGSSSKLWIYSTSNLASGVPARFSGSGSGTSYSLTISSMEAEDAASYFCHQWSSYPPTFGGGTKLEIKRADAAPTVSIFPPSSEQLTSGGASVVCFLNNFYPKDINVKWKIDGSERQNGVLNSWTDQDSKDSTYSMSSTLTLTKDEYERHNSYTCEATHKTSTSPIVKSFNRNEC

SEQ ID NO: 4 - protein, 467 aa, Artificial Sequence
  Heavy chain amino acid sequence
MEFGLSWVFLVALFRGVQCASQVQLQQPGAELVKPGASVNLSCKASGYTFTSYWMHWVKQRPGQGREWIGEINPRNGRTNYNEKFKSKATLTVDKSSSTAYMQLSSLTSEDSAVYCCARLSVGFAYWGQGTLVTVSAAKTTAPSVYPLAPVCGDTTGSSVTLGCLVKGYFPEPVTLTWNSGSLSSGVHTFPAVLQSDLYTLSSSVTVTSSTWPSQSITCNVAHPASSTKVDKKLEPRGPTIKPCPPCKCPAPNAAGGPSVFIFPPKIKDVLMISLSPIVTCVVVDVSEDDPDVQISWFVNNVEVHTAQTQTHREDYNSTLRVVSALPIQHQDWMSGKEFKCKVNNKDLGAPIERTISKPKGSVRAPQVYVLPPPEEEMTKKQVTLTCMVTDFMPEDIYVEWTNNGKTELNYKNTEPVLDSDGSYFMYSKLRVEKKNWVERNSYSCSVVHEGLHNHHTTKSFSRTPGK

SEQ ID NO: 5 - protein, 114 aa, Artificial Sequence
  Amino acid sequence of light chain variable region
QIVLTQSPVIMSASPGEKVTLTCSASSSVSSSYLYWYQQKPGSSSKLWIYSTSNLASGVPARFSGSGSGTSYSLTISSMEAEDAASYFCHQWSSYPPTFGGGTKLEIKRADAAP

SEQ ID NO: 6 - protein, 13 aa, Artificial Sequence
  Amino acid sequence of light chain CDR1
CSASSSVSSSYLY

SEQ ID NO: 7 - protein, 7 aa, Artificial Sequence
  Amino acid sequence of light chain CDR2
STSNLAS

SEQ ID NO: 8 - protein, 9 aa, Artificial Sequence
  Amino acid sequence of light chain CDR3
HQWSSYPPT

SEQ ID NO: 9 - protein, 126 aa, Artificial Sequence
  Amino acid sequence of heavy chain variable region
QVQLQQPGAELVKPGASVNLSCKASGYTFTSYWMHWVKQRPGQGREWIGEINPRNGRTNYNEKFKSKATLTVDKSSSTAYMQLSSLTSEDSAVYCCARLSVGFAYWGQGTLVTVSAAKTTAPSVYP

SEQ ID NO: 10 - protein, 5 aa, Artificial Sequence
  Amino acid sequence of heavy chain CDR1
SYWMH

SEQ ID NO: 11 - protein, 17 aa, Artificial Sequence
  Amino acid sequence of heavy chain CDR2
EINPRNGRTNYNEKFKS

SEQ ID NO: 12 - protein, 7 aa, Artificial Sequence
  Amino acid sequence of heavy chain CDR3
LSVGFAY

SEQ ID NO: 13 - DNA, 28 bp, Artificial Sequence
  Primer FSHR-F
gtttccacaaccatggccctgctcctgg

SEQ ID NO: 14 - DNA, 49 bp, Artificial Sequence
  Primer FSHR-R
ggttgattaactcgagttagttttgggctaaatgacttagagggacaag